European Patent Specification EP 3 398 612 B1, published July 29, 2026. Title: Stable Formulations of Antibodies to Human Programmed Death Receptor PD-1 and Related Treatments. Applicant: Merck Sharp & Dohme Corp. Sharma, Manoj K. Narasimhan, Chakravarthy Nachu Gergich, Kevin Kang, Soonmo Peter. The sequence listing filed with the application follows.

SEQUENCE LISTING (38 sequences)

SEQ ID NO: 1 - DNA, 435 bp, Artificial Sequence
  hPD-1.08A heavy chain variable region
atgrgatggagctgtatcatkctctttttggtagcaacagctacaggtgtccactcccaggtccaactgcagcagcctggggctgaactggtgaagcctggggcttcagtgaagttgtcctgcaaggcctctggctacaccttcaccagttattatctgtactggatgaaacagaggcctggacaaggccttgagtggattgggggggttaatcctagtaatggtggtactaacttcagtgagaagttcaagagcaaggccacactgactgtagacaaatcctccagcacagcctacatgcaactcagcagcctgacatctgaggactctgcggtctattactgtacaagaagggattctaactacgacgggggctttgactactggggccaaggcactactctcacagtctcctcagccaaaacgacaccccca

SEQ ID NO: 2 - DNA, 453 bp, Artificial Sequence
  hPD-1.08A light chain variable region
atggagacagacacactcctgctatgggtactgctgctctgggttccaggttccactggtgacattgtgctgacacagtctcctacttccttagctgtatctctggggcagagggccaccatctcatgcagggccagcaaaagtgtcagtacatctggctttagttatttgcactggtaccaacagaaaccaggacagccacccaaactcctcatctttcttgcatccaacctagagtctggggtccctgccaggttcagtggcagtgggtctgggacagacttcaccctcaacatccatcctgtggaggaggaggacgctgcaacctattattgtcagcacagttgggagcttccgctcacgttcggtgctgggaccaagctggagctgaaacgggctgatgctgcaccaactgtatccatcttcccaccatccagtaagcttgggaagggc

SEQ ID NO: 3 - DNA, 464 bp, Artificial Sequence
  hPD-1.09A heavy chain variable region
atgraatgcagctgggttatyctctttttggtagcaacagctacaggtgtccactcccaggtccaactgcagcagcctggggctgaactggtgaagcctgggacttcagtgaagttgtcctgcaaggcttctggctacaccttcaccaactactatatgtactgggtgaagcagaggcctggacaaggccttgagtggattggggggattaatcctagcaatggtggtactaacttcaatgagaagttcaagaacaaggccacactgactgtagacagttcctccagcacaacctacatgcaactcagcagcctgacatctgaggactctgcggtctattactgtacaagaagggattataggttcgacatgggctttgactactggggccaaggcaccactctcacagtctcctcagccaaaacgacacccccatccgtytatcccbtggcccctggaagctt

SEQ ID NO: 4 - DNA, 438 bp, Artificial Sequence
  hPD-1.09A light chain variable region
atggagwcagacacactsctgytatgggtactgctgctctgggttccaggttccactggcgacattgtgctgacacagtctcctgcttccttagctgtatctctgggacagagggccgccatctcatgcagggccagcaaaggtgtcagtacatctggctatagttatttgcactggtaccaacagaaaccaggacagtcacccaaactcctcatctatcttgcatcctacctagaatctggggtccctgccaggttcagtggcagtgggtctgggacagacttcaccctcaacatccatcctgtggaggaggaggatgctgcaacctattactgtcagcacagtagggaccttccgctcacgttcggtactgggaccaagctggagctgaaacgggctgatgctgcaccaactgtatccatcttcccaccatccagt

SEQ ID NO: 5 - protein, 122 aa, Artificial Sequence
  hPD-1.08A heavy chain variable region
QVQLQQPGAELVKPGASVKLSCKASGYTFTSYYLYWMKQRPGQGLEWIGGVNPSNGGTNFSEKFKSKATLTVDKSSSTAYMQLSSLTSEDSAVYYCTRRDSNYDGGFDYWGQGTTLTVSSAK

SEQ ID NO: 6 - protein, 111 aa, Artificial Sequence
  hPD-1.08A light chain variable region
DIVLTQSPTSLAVSLGQRATISCRASKSVSTSGFSYLHWYQQKPGQPPKLLIFLASNLESGVPARFSGSGSGTDFTLNIHPVEEEDAATYYCQHSWELPLTFGAGTKLELK

SEQ ID NO: 7 - protein, 122 aa, Artificial Sequence
  hPD-1.09A heavy chain variable region
QVQLQQPGAELVKPGTSVKLSCKASGYTFTNYYMYWVKQRPGQGLEWIGGINPSNGGTNFNEKFKNKATLTVDSSSSTTYMQLSSLTSEDSAVYYCTRRDYRFDMGFDYWGQGTTLTVSSAK

SEQ ID NO: 8 - protein, 111 aa, Artificial Sequence
  hPD-1.09A light chain variable region
DIVLTQSPASLAVSLGQRAAISCRASKGVSTSGYSYLHWYQQKPGQSPKLLIYLASYLESGVPARFSGSGSGTDFTLNIHPVEEEDAATYYCQHSRDLPLTFGTGTKLELK

SEQ ID NO: 9 - protein, 15 aa, Artificial Sequence
  hPD-1.08A light chain CDR1
RASKSVSTSGFSYLH

SEQ ID NO: 10 - protein, 7 aa, Artificial Sequence
  hPD-1.08A light chain CDR2
LASNLES

SEQ ID NO: 11 - protein, 9 aa, Artificial Sequence
  hPD-1-08A light chain CDR3
QHSWELPLT

SEQ ID NO: 12 - protein, 5 aa, Artificial Sequence
  hPD-1.08A heavy chain CDR1
SYYLY

SEQ ID NO: 13 - protein, 17 aa, Artificial Sequence
  hPD-1.08A heavy chain CDR2
GVNPSNGGTNFSEKFKS

SEQ ID NO: 14 - protein, 11 aa, Artificial Sequence
  hPD-1.08A heavy chain CDR3
RDSNYDGGFDY

SEQ ID NO: 15 - protein, 15 aa, Artificial Sequence
  hPD-1.09A light chain CDR1
RASKGVSTSGYSYLH

SEQ ID NO: 16 - protein, 7 aa, Artificial Sequence
  hPD-1.09A light chain CDR2
LASYLES

SEQ ID NO: 17 - protein, 9 aa, Artificial Sequence
  hPD-1.09A light chain CDR3
QHSRDLPLT

SEQ ID NO: 18 - protein, 5 aa, Artificial Sequence
  hPD-1.09A heavy chain CDR1
NYYMY

SEQ ID NO: 19 - protein, 17 aa, Artificial Sequence
  hPD-1.09A heavy chain CDR2
GINPSNGGTNFNEKFKN

SEQ ID NO: 20 - protein, 11 aa, Artificial Sequence
  hPD-1.09A heavy chain CDR3
RDYRFDMGFDY

SEQ ID NO: 21 - DNA, 417 bp, Artificial Sequence
  109A-H heavy chain variable region
  sig_peptide (1)..(57)
atggactggacctggagcatccttttcttggtggcagcaccaacaggagcccactcccaagtgcagctggtgcagtctggagttgaagtgaagaagcccggggcctcagtgaaggtctcctgcaaggcttctggctacacctttaccaactactatatgtactgggtgcgacaggcccctggacaagggcttgagtggatgggagggattaatcctagcaatggtggtactaacttcaatgagaagttcaagaacagagtcaccttgaccacagactcatccacgaccacagcctacatggaactgaagagcctgcaatttgacgacacggccgtttattactgtgcgagaagggattataggttcgacatgggctttgactactggggccaagggaccacggtcaccgtctcgagc

SEQ ID NO: 22 - DNA, 417 bp, Artificial Sequence
  Codon optimized 109A-H heavy chain variable region
  sig_peptide (1)..(57)
atggactggacctggtctatcctgttcctggtggccgctcctaccggcgctcactcccaggtgcagctggtgcagtccggcgtggaggtgaagaagcctggcgcctccgtcaaggtgtcctgcaaggcctccggctacaccttcaccaactactacatgtactgggtgcggcaggctcccggccagggactggagtggatgggcggcatcaacccttccaacggcggcaccaacttcaacgagaagttcaagaaccgggtgaccctgaccaccgactcctccaccaccaccgcctacatggagctgaagtccctgcagttcgacgacaccgccgtgtactactgcgccaggcgggactaccggttcgacatgggcttcgactactggggccagggcaccaccgtgaccgtgtcctcc

SEQ ID NO: 23 - DNA, 1398 bp, Artificial Sequence
  Codon optimized 409A-H heavy chain full length
  sig_peptide (1)..(57)
atggccgtgctgggcctgctgttctgcctggtgaccttcccttcctgcgtgctgtcccaggtgcagctggtgcagtccggcgtggaggtgaagaagcctggcgcctccgtcaaggtgtcctgtaaggcctccggctacaccttcaccaactactacatgtactgggtgcggcaggccccaggccagggactggagtggatgggcggcatcaacccttccaacggcggcaccaacttcaacgagaagttcaagaaccgggtgaccctgaccaccgactcctccaccacaaccgcctacatggaactgaagtccctgcagttcgacgacaccgccgtgtactactgcgccaggcgggactaccggttcgacatgggcttcgactactggggccagggcaccaccgtgaccgtgtcctccgctagcaccaagggcccttccgtgttccctctggccccttgctcccggtccacctccgagtccaccgccgctctgggctgtctggtgaaggactacttccctgagcctgtgaccgtgagctggaactctggcgccctgacctccggcgtgcacaccttccctgccgtgctgcagtcctccggcctgtactccctgtcctccgtggtgaccgtgccttcctcctccctgggcaccaagacctacacctgcaacgtggaccacaagccttccaacaccaaggtggacaagcgggtggagtccaagtacggccctccttgccctccctgccctgcccctgagttcctgggcggaccctccgtgttcctgttccctcctaagcctaaggacaccctgatgatctcccggacccctgaggtgacctgcgtggtggtggacgtgtcccaggaagatcctgaggtccagttcaattggtacgtggatggcgtggaggtgcacaacgccaagaccaagcctcgggaggaacagttcaactccacctaccgggtggtgtctgtgctgaccgtgctgcaccaggactggctgaacggcaaggaatacaagtgcaaggtcagcaacaagggcctgccctcctccatcgagaaaaccatctccaaggccaagggccagcctcgcgagcctcaggtgtacaccctgcctcctagccaggaagagatgaccaagaatcaggtgtccctgacatgcctggtgaagggcttctacccttccgatatcgccgtggagtgggagagcaacggccagccagagaacaactacaagaccacccctcctgtgctggactccgacggctccttcttcctgtactccaggctgaccgtggacaagtcccggtggcaggaaggcaacgtcttttcctgctccgtgatgcacgaggccctgcacaaccactacacccagaagtccctgtccctgtctctgggcaag

SEQ ID NO: 24 - DNA, 393 bp, Artificial Sequence
  K09A-L-11 light chain variable region
  sig_peptide (1)..(60)
atggaagccccagctcagcttctcttcctcctgctactctggctcccagataccaccggagaaattgtgttgacacagtctccagccaccctgtctttgtctccaggggaaagagccaccctctcctgcagggccagcaaaggtgtcagtacatctggctatagttatttgcactggtatcaacagaaacctggccaggctcccaggctcctcatctatcttgcatcctacctagaatctggcgtcccagccaggttcagtggtagtgggtctgggacagacttcactctcaccatcagcagcctagagcctgaagattttgcagtttattactgtcagcacagcagggaccttccgctcacgttcggcggagggaccaaagtggagatcaaa

SEQ ID NO: 25 - DNA, 393 bp, Artificial Sequence
  K09A-L-16 light chain variable region
  sig_peptide (1)..(60)
atggaaaccccagcgcagcttctcttcctcctgctactctggctcccagataccaccggagaaattgtgctgactcagtctccactctccctgcccgtcacccctggagagccggcctccatctcctgcagggccagcaaaggtgtcagtacatctggctatagttatttgcattggtacctccagaagccagggcagtctccacagctcctgatctatcttgcatcctacctagaatctggggtccctgacaggttcagtggcagtggatcaggcacagattttacactgaaaatcagcagagtggaggctgaggatgttggggtttattactgccagcatagtagggaccttccgctcacgtttggccaggggaccaagctggagatcaaa

SEQ ID NO: 26 - DNA, 393 bp, Artificial Sequence
  K09A-L-17 light chain variable region
  sig_peptide (1)..(60)
atgaggctccctgctcagctcctggggctgctaatgctctgggtctctggatccagtggggatattgtgatgacccagactccactctccctgcccgtcacccctggagagccggcctccatctcctgcagggccagcaaaggtgtcagtacatctggctatagttatttgcattggtatctgcagaagccagggcagtctccacagctcctgatctatcttgcatcctacctagaatctggagtcccagacaggttcagtggcagtgggtcaggcactgctttcacactgaaaatcagcagggtggaggctgaggatgttggactttattactgccagcatagtagggaccttccgctcacgtttggccaggggaccaagctggagatcaaa

SEQ ID NO: 27 - DNA, 390 bp, Artificial Sequence
  Codon optimized K09A-L-11 light chain variable region
  sig_peptide (1)..(57)
atggcccctgtgcagctgctgggcctgctggtgctgttcctgcctgccatgcggtgcgagatcgtgctgacccagtcccctgccaccctgtccctgagccctggcgagcgggctaccctgagctgcagagcctccaagggcgtgtccacctccggctactcctacctgcactggtatcagcagaagccaggccaggcccctcggctgctgatctacctggcctcctacctggagtccggcgtgcctgcccggttctccggctccggaagcggcaccgacttcaccctgaccatctcctccctggagcctgaggacttcgccgtgtactactgccagcactcccgggacctgcctctgacctttggcggcggaacaaaggtggagatcaag

SEQ ID NO: 28 - DNA, 390 bp, Artificial Sequence
  Codon optimized K09A-L-16 light chain variable region
  sig_peptide (1)..(57)
atggcccctgtgcagctgctgggcctgctggtgctgttcctgcctgccatgcggtgcgagatcgtgctgacccagtcccctctgtccctgcctgtgacccctggcgagcctgcctccatctcctgccgggcctccaagggcgtgtccacctccggctactcctacctgcactggtatctgcagaagcctggccagtccccccagctgctgatctacctggcctcctacctggagtccggcgtgcctgaccggttctccggctccggcagcggcaccgacttcaccctgaagatctcccgggtggaggccgaggacgtgggcgtgtactactgccagcactcccgggacctgcctctgaccttcggccagggcaccaagctggagatcaag

SEQ ID NO: 29 - DNA, 390 bp, Artificial Sequence
  Codon optimized K09A-L-17 light chain variable region
  sig_peptide (1)..(57)
atggcccctgtgcagctgctgggcctgctggtgctgttcctgcctgccatgcggtgcgacatcgtgatgacccagacccctctgtccctgcctgtgacccctggcgagcctgcctccatctcctgccgggcctccaagggcgtgtccacctccggctactcctacctgcactggtatctgcagaagcctggccagtcccctcagctgctgatctacctggcctcctacctggagtccggcgtgcctgaccggttctccggctccggaagcggcaccgcttttaccctgaagatctccagagtggaggccgaggacgtgggcctgtactactgccagcactcccgggacctgcctctgaccttcggccagggcaccaagctggagatcaag

SEQ ID NO: 30 - protein, 139 aa, Artificial Sequence
  109A-H heavy chain variable region
  sig_peptide (1)..(19)
MDWTWSILFLVAAPTGAHSQVQLVQSGVEVKKPGASVKVSCKASGYTFTNYYMYWVRQAPGQGLEWMGGINPSNGGTNFNEKFKNRVTLTTDSSTTTAYMELKSLQFDDTAVYYCARRDYRFDMGFDYWGQGTTVTVSS

SEQ ID NO: 31 - protein, 466 aa, Artificial Sequence
  409A-H heavy chain full length
  sig_peptide (1)..(19)
MAVLGLLFCLVTFPSCVLSQVQLVQSGVEVKKPGASVKVSCKASGYTFTNYYMYWVRQAPGQGLEWMGGINPSNGGTNFNEKFKNRVTLTTDSSTTTAYMELKSLQFDDTAVYYCARRDYRFDMGFDYWGQGTTVTVSSASTKGPSVFPLAPCSRSTSESTAALGCLVKDYFPEPVTVSWNSGALTSGVHTFPAVLQSSGLYSLSSVVTVPSSSLGTKTYTCNVDHKPSNTKVDKRVESKYGPPCPPCPAPEFLGGPSVFLFPPKPKDTLMISRTPEVTCVVVDVSQEDPEVQFNWYVDGVEVHNAKTKPREEQFNSTYRVVSVLTVLHQDWLNGKEYKCKVSNKGLPSSIEKTISKAKGQPREPQVYTLPPSQEEMTKNQVSLTCLVKGFYPSDIAVEWESNGQPENNYKTTPPVLDSDGSFFLYSRLTVDKSRWQEGNVFSCSVMHEALHNHYTQKSLSLSLGK

SEQ ID NO: 32 - protein, 130 aa, Artificial Sequence
  K09A-L-11 light chain variable region
  sig_peptide (1)..(19)
MAPVQLLGLLVLFLPAMRCEIVLTQSPATLSLSPGERATLSCRASKGVSTSGYSYLHWYQQKPGQAPRLLIYLASYLESGVPARFSGSGSGTDFTLTISSLEPEDFAVYYCQHSRDLPLTFGGGTKVEIK

SEQ ID NO: 33 - protein, 130 aa, Artificial Sequence
  K09A-L-16 light chain variable region
  sig_peptide (1)..(19)
MAPVQLLGLLVLFLPAMRCEIVLTQSPLSLPVTPGEPASISCRASKGVSTSGYSYLHWYLQKPGQSPQLLIYLASYLESGVPDRFSGSGSGTDFTLKISRVEAEDVGVYYCQHSRDLPLTFGQGTKLEIK

SEQ ID NO: 34 - protein, 130 aa, Artificial Sequence
  K09A-L-17 light chain variable region
  sig_peptide (1)..(19)
MAPVQLLGLLVLFLPAMRCDIVMTQTPLSLPVTPGEPASISCRASKGVSTSGYSYLHWYLQKPGQSPQLLIYLASYLESGVPDRFSGSGSGTAFTLKISRVEAEDVGLYYCQHSRDLPLTFGQGTKLEIK

SEQ ID NO: 35 - protein, 469 aa, Artificial Sequence
  109A-H heavy chain full length
  sig_peptide (1)..(19)
MAVLGLLFCLVTFPSCVLSQVQLVQSGVEVKKPGASVKVSCKASGYTFTNYYMYWVRQAPGQGLEWMGGINPSNGGTNFNEKFKNRVTLTTDSSTTTAYMELKSLQFDDTAVYYCARRDYRFDMGFDYWGQGTTVTVSSASTKGPSVFPLAPSSKSTSGGTAALGCLVKDYFPEPVTVSWNSGALTSGVHTFPAVLQSSGLYSLSSVVTVPSSSLGTQTYICNVNHKPSNTKVDKKVEPKSCDKTHTCPPCPAPELLGGPSVFLFPPKPKDTLMISRTPEVTCVVVDVSHEDPEVKFNWYVDGVEVHNAKTKPREEQYNSTYRVVSVLTVLHQDWLNGKEYKCKVSNKALPAPIEKTISKAKGQPREPQVYTLPPSRDELTKNQVSLTCLVKGFYPSDIAVEWESNGQPENNYKTTPPVLDSDGSFFLYSKLTVDKSRWQQGNVFSCSVMHEALHNHYTQKSLSLSPGK

SEQ ID NO: 36 - protein, 237 aa, Artificial Sequence
  K09A-L-11 light chain full length
  sig_peptide (1)..(19)
MAPVQLLGLLVLFLPAMRCEIVLTQSPATLSLSPGERATLSCRASKGVSTSGYSYLHWYQQKPGQAPRLLIYLASYLESGVPARFSGSGSGTDFTLTISSLEPEDFAVYYCQHSRDLPLTFGGGTKVEIKRTVAAPSVFIFPPSDEQLKSGTASVVCLLNNFYPREAKVQWKVDNALQSGNSQESVTEQDSKDSTYSLSSTLTLSKADYEKHKVYACEVTHQGLSSPVTKSFNRGEC

SEQ ID NO: 37 - protein, 237 aa, Artificial Sequence
  K09A-L-16 light chain full length
  sig_peptide (1)..(19)
MAPVQLLGLLVLFLPAMRCEIVLTQSPLSLPVTPGEPASISCRASKGVSTSGYSYLHWYLQKPGQSPQLLIYLASYLESGVPDRFSGSGSGTDFTLKISRVEAEDVGVYYCQHSRDLPLTFGQGTKLEIKRTVAAPSVFIFPPSDEQLKSGTASVVCLLNNFYPREAKVQWKVDNALQSGNSQESVTEQDSKDSTYSLSSTLTLSKADYEKHKVYACEVTHQGLSSPVTKSFNRGEC

SEQ ID NO: 38 - protein, 237 aa, Artificial Sequence
  K09A-L-17 light chain full length
  sig_peptide (1)..(19)
MAPVQLLGLLVLFLPAMRCDIVMTQTPLSLPVTPGEPASISCRASKGVSTSGYSYLHWYLQKPGQSPQLLIYLASYLESGVPDRFSGSGSGTAFTLKISRVEAEDVGLYYCQHSRDLPLTFGQGTKLEIKRTVAAPSVFIFPPSDEQLKSGTASVVCLLNNFYPREAKVQWKVDNALQSGNSQESVTEQDSKDSTYSLSSTLTLSKADYEKHKVYACEVTHQGLSSPVTKSFNRGEC